European Patent Application EP 4 541 815 A1, published April 23, 2025. Title: 抗乙型肝炎病毒的抗体及其制备和应用. Applicant: 华辉安健（北京）生物科技有限公司. Application CN. The sequence listing filed with the application follows.

SEQUENCE LISTING (39 sequences)

SEQ ID NO: 1 - protein, 120 aa, (Artificial Sequence)
QVQLQQSGPGLVKPSQTLSLTCAISGDSVSSNSAAWNWIRQSPSRGLEWLGRTYYRSKWYNDYAVSVKSRITINPDTSKNQFSLQLNSVTPEDTAVYYCARGTRWGMDVWGQGTLVTVSS

SEQ ID NO: 2 - protein, 330 aa, (Artificial Sequence)
ASTKGPSVFPLAPSSKSTSGGTAALGCLVKDYFPEPVTVSWNSGALTSGVHTFPAVLQSSGLYSLSSVVTVPSSSLGTQTYICNVNHKPSNTKVDKKVEPKSCDKTHTCPPCPAPELLAGPSVFLFPPKPKDTLMISRTPEVTCVVVDVSHEDPEVKFNWYVDGVEVHNAKTKPREEQYNSTYRVVSVLTVLHQDWLNGKEYKCKVSNKALPAPIEKTISKAKGQPREPQVYTLPPSRDELTKNQVSLTCLVKGFYPSDIAVEWESNGQPENNYKTTPPVLDSDGSFFLYSKLTVDKSRWQQGNVFSCSVLHEALHSHYTQKSLSLSPGK

SEQ ID NO: 3 - DNA, 360 bp, (Artificial Sequence)
  source 1..360: mol_type = other DNA
caggtacagctgcagcagtcaggtccaggactggtgaagccctcgcagaccctctcactcacctgtgccatctccggggacagtgtctctagcaacagtgctgcttggaactggatcaggcagtccccatcgagaggccttgagtggctgggaaggacatactacaggtccaagtggtataatgattatgcagtatctgtgaaaagtcgaataaccatcaacccagacacatccaagaaccagttctccctgcagctgaactctgtgactcccgaggacacggctgtgtattactgtgcaagaggaacacgttggggtatggacgtctggggccaagggaccctggtcaccgtctcttca

SEQ ID NO: 4 - DNA, 993 bp, (Artificial Sequence)
  source 1..993: mol_type = other DNA
gctagcaccaagggcccatcggtcttccccctggcaccctcctccaagagcacctctgggggcacagcggccctgggctgcctggtcaaggactacttccccgaaccggtgacggtgtcgtggaactcaggcgccctgaccagcggcgtgcacaccttcccggctgtcctacagtcctcaggactctactccctcagcagcgtggtgaccgtgccctccagcagcttgggcacccagacctacatctgcaacgtgaatcacaagcccagcaacaccaaggtggacaagaaggttgagcccaaatcttgtgacaaaactcacacatgcccaccgtgcccagcacctgaactcctggcgggaccgtcagtcttcctcttccccccaaaacccaaggacaccctcatgatctcccggacccctgaggtcacatgcgtggtggtggacgtgagccacgaagaccctgaggtcaagttcaactggtacgtggacggcgtggaggtgcataatgccaagacaaagccgcgggaggagcagtacaacagcacgtaccgtgtggtcagcgtcctcaccgtcctgcaccaggactggctgaatggcaaggagtacaagtgcaaggtctccaacaaagccctcccagcccccatcgagaaaaccatctccaaagccaaagggcagccccgagaaccacaggtgtacaccctgcccccatcccgggatgagctgaccaagaaccaggtcagcctgacctgcctggtcaaaggcttctatcccagcgacatcgccgtggagtgggagagcaatgggcagccggagaacaactacaagaccacgcctcccgtgctggactccgacggctccttcttcctctacagcaagctcaccgtggacaagagcaggtggcagcaggggaacgtcttctcatgctccgtgctgcatgaggctctgcacagccactacacgcagaagagcctctccctgtctccgggtaaatga

SEQ ID NO: 5 - protein, 110 aa, (Artificial Sequence)
QSVLTQPPSASGTPGQRVTISCSGSSSNIGSYYVYWYQQLPGTAPKLLIYGNNQRPSGVPDRFSGSKSGTSASLAITGLQAEDEADYYCQSYDSSLSGVIFGGGTKLTVL

SEQ ID NO: 6 - protein, 106 aa, (Artificial Sequence)
GQPKAAPSVTLFPPSSEELQANKATLVCLISDFYPGAVTVAWKADSSPVKAGVETTTPSKQSNNKYAASSYLSLTPEQWKSHRSYSCQVTHEGSTVEKTVAPTECS

SEQ ID NO: 7 - DNA, 330 bp, (Artificial Sequence)
  source 1..330: mol_type = other DNA
cagagcgtcctgacccagccacccagcgcaagcggcacccccggccagcgagtgaccatttcatgcagcggcagcagcagcaacattgggtcctactatgtgtactggtatcagcagctgcccggaacagctcctaagctgctgatctacggaaacaatcagcggccaagcggcgtccccgacagattctctggcagtaaatcagggactagcgcctccctggctatcaccggactgcaggcagaggacgaagccgattactattgccagtcttatgatagctccctgagtggggtgatttttggcgggggaactaaactgaccgtcctg

SEQ ID NO: 8 - DNA, 321 bp, (Artificial Sequence)
  source 1..321: mol_type = other DNA
ggtcagcccaaggctgccccctcggtcactctgttcccgccctcctctgaggagcttcaagccaacaaggccacactggtgtgtctcataagtgacttctacccgggagccgtgacagtggcctggaaggcagattccagccccgtcaaggcgggagtggagaccaccacaccctccaaacaaagcaacaacaagtacgcggccagcagctatctgagcctgacgcctgagcagtggaagtcccacagaagctacagctgccaggtcacgcatgaagggagcaccgtggagaagacagtggcccctacagaatgttcatga

SEQ ID NO: 9 - DNA, 23 bp, (Artificial Sequence)
  source 1..23: mol_type = other DNA
attccaagatgagtgttcgctgg

SEQ ID NO: 10 - DNA, 23 bp, (Artificial Sequence)
  source 1..23: mol_type = other DNA
ctcgtacaagtcgatctgcgagg

SEQ ID NO: 11 - DNA, 25 bp, (Artificial Sequence)
  source 1..25: mol_type = other DNA
caccgattccaagatgagtgttcgc

SEQ ID NO: 12 - DNA, 25 bp, (Artificial Sequence)
  source 1..25: mol_type = other DNA
aaacgcgaacactcatcttggaatc

SEQ ID NO: 13 - DNA, 25 bp, (Artificial Sequence)
  source 1..25: mol_type = other DNA
caccgctcgtacaagtcgatctgcg

SEQ ID NO: 14 - DNA, 25 bp, (Artificial Sequence)
  source 1..25: mol_type = other DNA
aaaccgcagatcgacttgtacgagc

SEQ ID NO: 15 - DNA, 27 bp, (Artificial Sequence)
  source 1..27: mol_type = other DNA
cctacttgagggtgaaaggtgggagga

SEQ ID NO: 16 - DNA, 26 bp, (Artificial Sequence)
  source 1..26: mol_type = other DNA
agtatgttccatgaaggtctacctag

SEQ ID NO: 17 - DNA, 26 bp, (Artificial Sequence)
  source 1..26: mol_type = other DNA
ggtggatgtataaggaataccatgtg

SEQ ID NO: 18 - DNA, 30 bp, (Artificial Sequence)
  source 1..30: mol_type = other DNA
ggagaactggagacagtaatagagcactac

SEQ ID NO: 19 - DNA, 23 bp, (Artificial Sequence)
  source 1..23: mol_type = other DNA
attccaagatgagtgttcgctgg

SEQ ID NO: 20 - DNA, 23 bp, (Artificial Sequence)
  source 1..23: mol_type = other DNA
ctctcaggagtcgatctgcaagg

SEQ ID NO: 21 - DNA, 23 bp, (Artificial Sequence)
  source 1..23: mol_type = other DNA
acttgatccgtccacaaccttgg

SEQ ID NO: 22 - DNA, 23 bp, (Artificial Sequence)
  source 1..23: mol_type = other DNA
ctttgtcagtgcgtctgacatgg

SEQ ID NO: 23 - DNA, 40 bp, (Artificial Sequence)
  source 1..40: mol_type = other DNA
ttaatacgactcactataggctctcaggagtcgatctgca

SEQ ID NO: 24 - DNA, 40 bp, (Artificial Sequence)
  source 1..40: mol_type = other DNA
gctatttctagctctaaaactgcagatcgactcctgagag

SEQ ID NO: 25 - DNA, 36 bp, (Artificial Sequence)
  source 1..36: mol_type = other DNA
gttttagagctagaaatagcaagttaaaataaggct

SEQ ID NO: 26 - DNA, 38 bp, (Artificial Sequence)
  source 1..38: mol_type = other DNA
tttttcaagttgataacggactagccttattttaactt

SEQ ID NO: 27 - DNA, 32 bp, (Artificial Sequence)
  source 1..32: mol_type = other DNA
gttatcaacttgaaaaagtggcaccgagtcgg

SEQ ID NO: 28 - DNA, 25 bp, (Artificial Sequence)
  source 1..25: mol_type = other DNA
aaaaaaagcaccgactcggtgccac

SEQ ID NO: 29 - DNA, 27 bp, (Artificial Sequence)
  source 1..27: mol_type = other DNA
agagttgctgtgaaggtacaagtactc

SEQ ID NO: 30 - DNA, 27 bp, (Artificial Sequence)
  source 1..27: mol_type = other DNA
atttgctctgctgccctaactgaacaa

SEQ ID NO: 31 - protein, 330 aa, (Artificial Sequence) [sequence omitted]

SEQ ID NO: 32 - protein, 7 aa, (Artificial Sequence)
SNSAAWN

SEQ ID NO: 33 - protein, 15 aa, (Artificial Sequence)
RTYYRSKWYNDYAVS

SEQ ID NO: 34 - protein, 8 aa, (Artificial Sequence)
GTRWGMDV

SEQ ID NO: 35 - protein, 15 aa, (Artificial Sequence)
SGSSSNIGSYYVYWY

SEQ ID NO: 36 - protein, 7 aa, (Artificial Sequence)
GNNQRPS

SEQ ID NO: 37 - protein, 11 aa, (Artificial Sequence)
QSYDSSLSGVI

SEQ ID NO: 38 - protein, 330 aa, (Artificial Sequence) [sequence omitted]

SEQ ID NO: 39 - DNA, 123 bp, (Artificial Sequence)
  source 1..123: mol_type = other DNA
ttaatacgactcactataggctctcaggagtcgatctgcagttttagagctagaaatagcaagttaaaataaggctagtccgttatcaacttgaaaaagtggcaccgagtcggtgcttttttt